European Patent Application EP 4 159 747 A1, published April 5, 2023. Title: Composition for neutralizing coronavirus. Applicant: Bio3S. The sequence listing filed with the application follows.

SEQUENCE LISTING (1 sequence)

SEQ ID NO: 1 - protein, 193 aa, Artificial Sequence
  truncated Concanavalin A
ELDTYPNTDIGDPSYPHIGIDIKSVRSKKTAKWNMQDGKVGTAHIIYNSVDKRLSAVVSYPNADATSVSYDVDLNDVLPEWVRVGLSASTGLYKETNTILSWSFTSKLKSNSTHQTDALHFMFNQFSKDQKDLILQGDATTGTDGNLELTRVSSNGSPEGSSVGRALFYAPVHIWESSATVSAFEATFAFLIK